European Patent Application EP 4 269 590 A1, published November 1, 2023. Title: Immunoglobulin binding polypeptide. Applicant: ProteNova Co., Ltd. The sequence listing filed with the application follows.

SEQUENCE LISTING (16 sequences)

SEQ ID NO: 1 - protein, 58 aa, Staphylococcus aureus
ADNKFNKEQQNAFYEILHLPNLTEEQRNGFIQSLKDDPSVSKEILAEAKKLNDAQAPK

SEQ ID NO: 2 - protein, 58 aa, Artificial Sequence
  Modified domain C
ADNAFNTEQQNAFYEILHLPNLTEEQRNAFIQSLRDDPSKSKKILKEAKKLNKAQAPK

SEQ ID NO: 3 - protein, 58 aa, Artificial Sequence
  Modified domain C
ADNAFNTEQQNAFYEILHLPNLTEEQRNAFIQSLRDDPSVSAEILAEARRLNDAQAPR

SEQ ID NO: 4 - protein, 58 aa, Staphylococcus aureus
ADNNFNKEQQNAFYEILNMPNLNEEQRNGFIQSLKDDPSQSANLLSEAKKLNESQAPK

SEQ ID NO: 5 - protein, 58 aa, Artificial Sequence
  Modified domain A
ADNAFNTEQQNAFYEILNMPNLNEEQRNGFIQSLRDDPSKSAKLLKEAKKLNKSQAPK

SEQ ID NO: 6 - protein, 58 aa, Artificial Sequence
  Modified domain A
ADNAFNTEQQNAFYEILNMPNLNEEQRNGFIQSLRDDPSQSANLLSEARRLNESQAPR

SEQ ID NO: 7 - protein, 58 aa, Staphylococcus aureus [sequence omitted]

SEQ ID NO: 8 - protein, 58 aa, Artificial Sequence
  Modified domain B
ADNAFNTEQQNAFYEILHLPNLNEEQRNGFIQSLRDDPSKSAKLLKEAKKLNKAQAPK

SEQ ID NO: 9 - protein, 58 aa, Artificial Sequence
  Modified domain B
ADNAFNTEQQNAFYEILHLPNLNEEQRNGFIQSLRDDPSQSANLLAEARRLNDAQAPR

SEQ ID NO: 10 - protein, 58 aa, Staphylococcus aureus
QQNNFNKDQQSAFYEILNMPNLNEAQRNGFIQSLKDDPSQSTNVLGEAKKLNESQAPK

SEQ ID NO: 11 - protein, 58 aa, Artificial Sequence
  Modified domain D
QQNAFNTDQQSAFYEILNMPNLNEAQRNGFIQSLRDDPSKSTKVLKEAKKLNKSQAPK

SEQ ID NO: 12 - protein, 58 aa, Artificial Sequence
  Modified domain D
QQNAFNTDQQSAFYEILNMPNLNEAQRNGFIQSLRDDPSQSANVLGEARRLNESQAPR

SEQ ID NO: 13 - protein, 58 aa, Staphylococcus aureus
NAAQHDEAQQNAFYQVLNMPNLNADQRNGFIQSLKDDPSQSANVLGEAQKLNDSQAPK

SEQ ID NO: 14 - protein, 58 aa, Artificial Sequence
  Modified domain E
NAAAHDTAQQNAFYQVLNMPNLNADQRNGFIQSLRDDPSKSAKVLKEAQKLNKSQAPK

SEQ ID NO: 15 - protein, 58 aa, Artificial Sequence
  Modified domain E
NAAAHDTAQQNAFYQVLNMPNLNADQRNGFIQSLRDDPSQSANVLGEARRLNDSQAPR

SEQ ID NO: 16 - DNA, 1921 bp, Staphylococcus aureus
tcgaaatagcgtgattttgcggttttaagccttttacttcctgaataaatctttcagcaaaatatttattttataagttgtaaaacttacctttaaatttaattataaatatagattttagtattgcaatacataattcgttatattatgatgactttacaaatacatacagggggtattaatttgaaaaagaaaaacatttattcaattcgtaaactaggtgtaggtattgcatctgtaactttaggtacattacttatatctggtggcgtaacacctgctgcaaatgctgcgcaacacgatgaagctcaacaaaatgctttttatcaagtcttaaatatgcctaacttaaatgctgatcaacgcaatggttttatccaaagccttaaagatgatccaagccaaagtgctaacgttttaggtgaagctcaaaaacttaatgactctcaagctccaaaagctgatgcgcaacaaaataacttcaacaaagatcaacaaagcgccttctatgaaatcttgaacatgcctaacttaaacgaagcgcaacgtaacggcttcattcaaagtcttaaagacgacccaagccaaagcactaacgttttaggtgaagctaaaaaattaaacgaatctcaagcaccgaaagctgataacaatttcaacaaagaacaacaaaatgctttctatgaaatcttgaatatgcctaacttaaacgaagaacaacgcaatggtttcatccaaagcttaaaagatgacccaagccaaagtgctaacctattgtcagaagctaaaaagttaaatgaatctcaagcaccgaaagcggataacaaattcaacaaagaacaacaaaatgctttctatgaaatcttacatttacctaacttaaacgaagaacaacgcaatggtttcatccaaagcctaaaagatgacccaagccaaagcgctaaccttttagcagaagctaaaaagctaaatgatgctcaagcaccaaaagctgacaacaaattcaacaaagaacaacaaaatgctttctatgaaattttacatttacctaacttaactgaagaacaacgtaacggcttcatccaaagccttaaagacgatccttcggtgagcaaagaaattttagcagaagctaaaaagctaaacgatgctcaagcaccaaaagaggaagacaataacaagcctggcaaagaagacaataacaagcctggcaaagaagacaataacaagcctggcaaagaagacaacaacaagcctggcaaagaagacaacaacaagcctggtaaagaagacaacaacaagcctggcaaagaagacggcaacaagcctggtaaagaagacaacaaaaaacctggtaaagaagatggcaacaagcctggtaaagaagacaacaaaaaacctggtaaagaagacggcaacaagcctggcaaagaagatggcaacaaacctggtaaagaagatggtaacggagtacatgtcgttaaacctggtgatacagtaaatgacattgcaaaagcaaacggcactactgctgacaaaattgctgcagataacaaattagctgataaaaacatgatcaaacctggtcaagaacttgttgttgataagaagcaaccagcaaaccatgcagatgctaacaaagctcaagcattaccagaaactggcgaagaaaatccattcatcggtacaactgtatttggtggattatcattagccttaggtgcagcgttattagctggacgtcgtcgcgaactataaaaacaaacaatacacaacgatagatatcattttatgcaaaccaattttaacttatatacgttgattaacacattcttatttgaaatgataagaatcatctaaatgcacgagcaacatcttttgttgctcagtgcattttttattttacttacttttctaaaca